European Patent Specification EP 3 515 435 B1, published February 25, 2026. Title: WASP-PROTECTING SMALL MOLECULES, COMPOSITIONS, METHODS AND USES THEREOF IN THE TREATMENT OF INNATE AND ACQUIRED IMMUNE-RELATED DISORDERS OR CONDITIONS. Applicant: Bar Ilan University. The sequence listing filed with the application follows.

SEQUENCE LISTING (18 sequences)

SEQ ID NO: 1 - protein, 502 aa, Homo sapiens
MSGGPMGGRPGGRGAPAVQQNIPSTLLQDHENQQLFEMLGRKCLTLATAVVQLYLALPPGAEHWTKEHCGAVCFVKDNPQKSYFIRLYGLQAGRLLWEQELYSQLVYSTPTPFFHTFAGDDCQAGLNFADEDEAQAFRALVQEKIQKRNQRQSGDRRQLPPPPTPANEERRGGLPPLPLHPGGDQGGPPVGPLSLGLATVDIQNPDITSSRYRGLPAPGPSPADKKRSGRKKISKADIGAPSGFKHVSHVGWDPQNGFDVNNLDPDLRSLFSRAGISEAQLTDAETSKLIYDFIEDQGGLEAVRQEMRRQEPLPPPPPPSRGGNQLPRPPIVGGNKGRSGPLPPVPLGIAPPPPTPRGPPPPGRGGPPPPPPPATGRSGPLPPPPPGAGGPPMPPPPPPPPPPPSSGNGPAPPPLPPALVPAGGLAPGGGRGALLDQIRQGIQLNKTPGAPESSALQPPPQSSEGLVGALMHVMQKRSRAIHSSDEGEDQAGDEDEDDEWDD

SEQ ID NO: 2 - DNA, 1509 bp, Homo sapiens
atgagtgggggcccaatgggaggaaggcccgggggccgaggagcaccagcggttcagcagaacataccctccaccctcctccaggaccacgagaaccagcaactctttgagatgcttggacgaaaatgcttgacgctggccactgcagttgttcagctgtacctggcgctgccccctggagctgagcactggaccaaggagcattgtggggctgtgtgcttcgtgaaggataacccccagaagtcctacttcatccgcctttacggccttcaggctggtcggctgctctgggaacaggagctgtactcacagcttgtctactccacccccacccccttcttccacaccttcgctggagatgactgccaagcggggctgaactttgcagacgaggacgaggcccaggccttccgggccctcgtgcaggagaagatacaaaaaaggaatcagaggcaaagtggagacagacgccagctacccccaccaccaacaccagccaatgaagagagaagaggagggctcccacccctgcccctgcatccaggtggagaccaaggaggccctccagtgggtccgctctccctggggctggcgacagtggacatccagaaccctgacatcacgagttcacgataccgtgggctcccagcacctggacctagcccagctgataagaaacgctcagggaggaagaagatcagcaaagctgatattggtgcacccagtggattcaagcatgtcagccacgtggggtgggacccccagaatggatttgacgtgaacaacctcgacccagatctgcggagtctgttctccagggcaggaatcagcgaggcccagctcaccgacgccgagacctctaaacttatctacgacttcattgaggaccagggtgggctggaggctgtgcggcaggagatgaggcgccaggagccacttccgccgcccccaccgccatctcgaggagggaaccagctcccccggccccctattgtggggggtaacaagggtcgttctggtccactgccccctgtacctttggggattgccccacccccaccaacaccccggggacccccacccccaggccgagggggccctccaccaccaccccctccagctactggacgttctggaccactgccccctccaccccctggagctggtgggccacccatgccaccaccaccgccaccaccgccaccgccgcccagctccgggaatggaccagcccctcccccactccctcctgctctggtgcctgccgggggcctggcccctggtgggggtcggggagcgcttttggatcaaatccggcagggaattcagctgaacaagacccctggggccccagagagctcagcgctgcagccaccacctcagagctcagagggactggtgggggccctgatgcacgtgatgcagaagagaagcagagccatccactcctccgacgaaggggaggaccaggctggcgatgaagatgaagatgatgaatgggatgactag

SEQ ID NO: 3 - RNA, 25 nt, Artificial Sequence
  HUMAN PKC theta RNA SEQUENCE
gagucuccguuggaugagguggaua

SEQ ID NO: 4 - RNA, 25 nt, Artificial Sequence
  HUMAN PKC theta RNA SEQUENCE
gcauccguuucugacgcacauguuu

SEQ ID NO: 5 - RNA, 25 nt, Artificial Sequence
  HUMAN PKC theta RNA SEQUENCE
ccggccgaaagugaaaucaccauuu

SEQ ID NO: 6 - RNA, 19 nt, Artificial Sequence
  NONSPECIFIC siRNA
uagcgacuaaacacaucaa

SEQ ID NO: 7 - RNA, 19 nt, Artificial Sequence
  NONSPECIFIC siRNA
uaaggcuaugaagagauac

SEQ ID NO: 8 - RNA, 19 nt, Artificial Sequence
  NONSPECIFIC siRNA
auguauuggccuguauuag

SEQ ID NO: 9 - RNA, 19 nt, Artificial Sequence
  NONSPECIFIC siRNA
augaacgugaauugcucaa

SEQ ID NO: 10 - RNA, 19 nt, Artificial Sequence
  NONSPECIFIC siRNA
ugguuuacaugucgacuaa

SEQ ID NO: 11 - DNA, 26 bp, Artificial Sequence
  RNA guide
aaactcgctggagatgtaagtggatc

SEQ ID NO: 12 - DNA, 25 bp, Artificial Sequence
  RNA guide
caccgatcacttacatctccagcga

SEQ ID NO: 13 - protein, 502 aa, Artificial Sequence
  Human WASp mutant R86C
MSGGPMGGRPGGRGAPAVQQNIPSTLLQDHENQQLFEMLGRKCLTLATAVVQLYLALPPGAEHWTKEHCGAVCFVKDNPQKSYFICLYGLQAGRLLWEQELYSQLVYSTPTPFFHTFAGDDCQAGLNFADEDEAQAFRALVQEKIQKRNQRQSGDRRQLPPPPTPANEERRGGLPPLPLHPGGDQGGPPVGPLSLGLATVDIQNPDITSSRYRGLPAPGPSPADKKRSGRKKISKADIGAPSGFKHVSHVGWDPQNGFDVNNLDPDLRSLFSRAGISEAQLTDAETSKLIYDFIEDQGGLEAVRQEMRRQEPLPPPPPPSRGGNQLPRPPIVGGNKGRSGPLPPVPLGIAPPPPTPRGPPPPGRGGPPPPPPPATGRSGPLPPPPPGAGGPPMPPPPPPPPPPPSSGNGPAPPPLPPALVPAGGLAPGGGRGALLDQIRQGIQLNKTPGAPESSALQPPPQSSEGLVGALMHVMQKRSRAIHSSDEGEDQAGDEDEDDEWDD

SEQ ID NO: 14 - DNA, 1509 bp, Artificial Sequence
  Human WASp mutant R86C
atgagtgggggcccaatgggaggaaggcccgggggccgaggagcaccagcggttcagcagaacataccctccaccctcctccaggaccacgagaaccagcaactctttgagatgcttggacgaaaatgcttgacgctggccactgcagttgttcagctgtacctggcgctgccccctggagctgagcactggaccaaggagcattgtggggctgtgtgcttcgtgaaggataacccccagaagtcctacttcatctgcctttacggccttcaggctggtcggctgctctgggaacaggagctgtactcacagcttgtctactccacccccacccccttcttccacaccttcgctggagatgactgccaagcggggctgaactttgcagacgaggacgaggcccaggccttccgggccctcgtgcaggagaagatacaaaaaaggaatcagaggcaaagtggagacagacgccagctacccccaccaccaacaccagccaatgaagagagaagaggagggctcccacccctgcccctgcatccaggtggagaccaaggaggccctccagtgggtccgctctccctggggctggcgacagtggacatccagaaccctgacatcacgagttcacgataccgtgggctcccagcacctggacctagcccagctgataagaaacgctcagggaggaagaagatcagcaaagctgatattggtgcacccagtggattcaagcatgtcagccacgtggggtgggacccccagaatggatttgacgtgaacaacctcgacccagatctgcggagtctgttctccagggcaggaatcagcgaggcccagctcaccgacgccgagacctctaaacttatctacgacttcattgaggaccagggtgggctggaggctgtgcggcaggagatgaggcgccaggagccacttccgccgcccccaccgccatctcgaggagggaaccagctcccccggccccctattgtggggggtaacaagggtcgttctggtccactgccccctgtacctttggggattgccccacccccaccaacaccccggggacccccacccccaggccgagggggccctccaccaccaccccctccagctactggacgttctggaccactgccccctccaccccctggagctggtgggccacccatgccaccaccaccgccaccaccgccaccgccgcccagctccgggaatggaccagcccctcccccactccctcctgctctggtgcctgccgggggcctggcccctggtgggggtcggggagcgcttttggatcaaatccggcagggaattcagctgaacaagacccctggggccccagagagctcagcgctgcagccaccacctcagagctcagagggactggtgggggccctgatgcacgtgatgcagaagagaagcagagccatccactcctccgacgaaggggaggaccaggctggcgatgaagatgaagatgatgaatgggatgactag

SEQ ID NO: 15 - protein, 502 aa, Artificial Sequence
  Human WASp mutant Y107C
MSGGPMGGRPGGRGAPAVQQNIPSTLLQDHENQQLFEMLGRKCLTLATAVVQLYLALPPGAEHWTKEHCGAVCFVKDNPQKSYFIRLYGLQAGRLLWEQELYSQLVCSTPTPFFHTFAGDDCQAGLNFADEDEAQAFRALVQEKIQKRNQRQSGDRRQLPPPPTPANEERRGGLPPLPLHPGGDQGGPPVGPLSLGLATVDIQNPDITSSRYRGLPAPGPSPADKKRSGRKKISKADIGAPSGFKHVSHVGWDPQNGFDVNNLDPDLRSLFSRAGISEAQLTDAETSKLIYDFIEDQGGLEAVRQEMRRQEPLPPPPPPSRGGNQLPRPPIVGGNKGRSGPLPPVPLGIAPPPPTPRGPPPPGRGGPPPPPPPATGRSGPLPPPPPGAGGPPMPPPPPPPPPPPSSGNGPAPPPLPPALVPAGGLAPGGGRGALLDQIRQGIQLNKTPGAPESSALQPPPQSSEGLVGALMHVMQKRSRAIHSSDEGEDQAGDEDEDDEWDD

SEQ ID NO: 16 - DNA, 1509 bp, Artificial Sequence
  Human WASp mutant Y107C
atgagtgggggcccaatgggaggaaggcccgggggccgaggagcaccagcggttcagcagaacataccctccaccctcctccaggaccacgagaaccagcaactctttgagatgcttggacgaaaatgcttgacgctggccactgcagttgttcagctgtacctggcgctgccccctggagctgagcactggaccaaggagcattgtggggctgtgtgcttcgtgaaggataacccccagaagtcctacttcatccgcctttacggccttcaggctggtcggctgctctgggaacaggagctgtactcacagcttgtctgctccacccccacccccttcttccacaccttcgctggagatgactgccaagcggggctgaactttgcagacgaggacgaggcccaggccttccgggccctcgtgcaggagaagatacaaaaaaggaatcagaggcaaagtggagacagacgccagctacccccaccaccaacaccagccaatgaagagagaagaggagggctcccacccctgcccctgcatccaggtggagaccaaggaggccctccagtgggtccgctctccctggggctggcgacagtggacatccagaaccctgacatcacgagttcacgataccgtgggctcccagcacctggacctagcccagctgataagaaacgctcagggaggaagaagatcagcaaagctgatattggtgcacccagtggattcaagcatgtcagccacgtggggtgggacccccagaatggatttgacgtgaacaacctcgacccagatctgcggagtctgttctccagggcaggaatcagcgaggcccagctcaccgacgccgagacctctaaacttatctacgacttcattgaggaccagggtgggctggaggctgtgcggcaggagatgaggcgccaggagccacttccgccgcccccaccgccatctcgaggagggaaccagctcccccggccccctattgtggggggtaacaagggtcgttctggtccactgccccctgtacctttggggattgccccacccccaccaacaccccggggacccccacccccaggccgagggggccctccaccaccaccccctccagctactggacgttctggaccactgccccctccaccccctggagctggtgggccacccatgccaccaccaccgccaccaccgccaccgccgcccagctccgggaatggaccagcccctcccccactccctcctgctctggtgcctgccgggggcctggcccctggtgggggtcggggagcgcttttggatcaaatccggcagggaattcagctgaacaagacccctggggccccagagagctcagcgctgcagccaccacctcagagctcagagggactggtgggggccctgatgcacgtgatgcagaagagaagcagagccatccactcctccgacgaaggggaggaccaggctggcgatgaagatgaagatgatgaatgggatgactag

SEQ ID NO: 17 - protein, 499 aa, Artificial Sequence
  Human WASp mutant A134T
MSGGPMGGRPGGRGAPAVQQNIPSTLLQDHENQQLFEMLGRKCLTLATAVVQLYLALPPGAEHWTKEHCGAVCFVKDNPQKSYFIRLYGLQAGRLLWEQELYSQLVYSTPTPFFHTFAGDDCQAGLNFADEDETQRALVQEKIQKRNQRQSGDRRQLPPPPTPANEERRGGLPPLPLHPGGDQGGPPVGPLSLGLATVDIQNPDITSSRYRGLPAPGPSPADKKRSGRKKISKADIGAPSGFKHVSHVGWDPQNGFDVNNLDPDLRSLFSRAGISEAQLTDAETSKLIYDFIEDQGGLEAVRQEMRRQEPLPPPPPPSRGGNQLPRPPIVGGNKGRSGPLPPVPGIAPPPPTPRGPPPPGRGGPPPPPPPATGRSGPLPPPPPGAGGPPMPPPPPPPPPPPSSGNGPAPPPLPPALVPAGGLAPGGGRGALLDQIRQGIQLNKTPGAPESSALQPPPQSSEGLVGALMHVMQKRSRAIHSSDEGEDQAGDEDEDDEWDD

SEQ ID NO: 18 - DNA, 1509 bp, Artificial Sequence
  Human WASp mutant A134T
atgagtgggggcccaatgggaggaaggcccgggggccgaggagcaccagcggttcagcagaacataccctccaccctcctccaggaccacgagaaccagcaactctttgagatgcttggacgaaaatgcttgacgctggccactgcagttgttcagctgtacctggcgctgccccctggagctgagcactggaccaaggagcattgtggggctgtgtgcttcgtgaaggataacccccagaagtcctacttcatccgcctttacggccttcaggctggtcggctgctctgggaacaggagctgtactcacagcttgtctactccacccccacccccttcttccacaccttcgctggagatgactgccaagcggggctgaactttgcagacgaggacgagacccaggccttccgggccctcgtgcaggagaagatacaaaaaaggaatcagaggcaaagtggagacagacgccagctacccccaccaccaacaccagccaatgaagagagaagaggagggctcccacccctgcccctgcatccaggtggagaccaaggaggccctccagtgggtccgctctccctggggctggcgacagtggacatccagaaccctgacatcacgagttcacgataccgtgggctcccagcacctggacctagcccagctgataagaaacgctcagggaggaagaagatcagcaaagctgatattggtgcacccagtggattcaagcatgtcagccacgtggggtgggacccccagaatggatttgacgtgaacaacctcgacccagatctgcggagtctgttctccagggcaggaatcagcgaggcccagctcaccgacgccgagacctctaaacttatctacgacttcattgaggaccagggtgggctggaggctgtgcggcaggagatgaggcgccaggagccacttccgccgcccccaccgccatctcgaggagggaaccagctcccccggccccctattgtggggggtaacaagggtcgttctggtccactgccccctgtacctttggggattgccccacccccaccaacaccccggggacccccacccccaggccgagggggccctccaccaccaccccctccagctactggacgttctggaccactgccccctccaccccctggagctggtgggccacccatgccaccaccaccgccaccaccgccaccgccgcccagctccgggaatggaccagcccctcccccactccctcctgctctggtgcctgccgggggcctggcccctggtgggggtcggggagcgcttttggatcaaatccggcagggaattcagctgaacaagacccctggggccccagagagctcagcgctgcagccaccacctcagagctcagagggactggtgggggccctgatgcacgtgatgcagaagagaagcagagccatccactcctccgacgaaggggaggaccaggctggcgatgaagatgaagatgatgaatgggatgactag